European Patent Specification EP 3 534 942 B1, published October 16, 2024. Title: ANTIGENS FOR DETECTING CHRONIC TOXOPLASMA INFECTION BY MONITORING CELLULAR IMMUNITY. Applicant: Sibley, Laurence David Brown, Kevin Wang, Quiling Saraav, Iti. The sequence listing filed with the application follows.

SEQUENCE LISTING (64 sequences)

SEQ ID NO: 1 - protein, 456 aa, Toxopolasmosis gondii
MGQALFLTVLLPVLFGVGPEAYGEASHSHSPASGRYIQQMLDQRCQEIAAELCQGGLRKMCVPSSRIVARNAVGITHQNTLEWRCFDTASLLESNQENNGVNCVDDCGHTIPCPGGVHRQNSNHATRHEILSKLVEEGVQRFCSPYQASANKYCNDKFPGTIARRSKGFGNNVEVAWRCYEKASLLYSVYAECASNCGTTWYCPGGRRGTSTELDKRHYTEEEGIRQAIGSVDSPCSEVEVCLPKDENPPVCLDESGQISRTGGGPPSQPPEMQQPADRSDERGGGKEQSPGGEAQPDHPTKGGNIDLPEKSTSPEKTPKTEIHGDSTKATLEEGQQLTLTFISTKLDVAVGSCHSLVANFLDGFLKFQTGSNSAFDVVEVEEPAGPAVLTIGLGHKGRLAVVLDYTRLNAALGSAAYVVEDSGCSSSEEVSFQGVGSGATLVVTTLGESPTAVSA

SEQ ID NO: 2 - protein, 321 aa, Toxopolasmosis gondii
MAYGEASHSHSPASGRYIQQMLDQRCQEIAAELCQGGLRKMCVPSSRIVARNAVGITHQNTLEWRCFDTASLLESNQENNGVNCVDDCGHTIPCPGGVHRQNSNHATRHEILSKLVEEGVQRFCSPYQASANKYCNDKFPGTIARRSKGFGNNVEVAWRCYEKASLLYSVYAECASNCGTTWYCPGGRRGTSTELDKRHYTEEEGIRQAIGSVDSPCSEVEVCLPKDENPPVCLDESGQISRTGGGPPSQPPEMQQPADRSDERGGGKEQSPGGEAQPDHPTKGGNIDLPEKSTSPEKTPKTEIHGDSTKATLEEGQQLTL

SEQ ID NO: 3 - DNA, 1920 bp, Toxopolasmosis gondii
acctgaaagcgggtgccgcgtcgctaccgtttcctgtggcgtctctagtgcgacatccgaagtaacagtaacgtccggcatggaacgccgacgcgggtgttccagtcgcctggctccttctactcgcacttcgatgttacgttccttattggtgcgacgcggttctcgtgttgctagacgtcgcaccggctgaaagctgtagaaaatttagttattttcctgtcagctagcttgcaggagtgcgtttttgtgtgttggtttcgtctcacatggctgctgatctgttgatgcagctgtgtacacgtgcctcgattctgtagttgacctagaacggatttgcaaagatgggccaggcgttgtttctcaccgttctattgccggtgttatttggcgttgggccagaagcatatggagaagcgtcgcattctcattcgccggcatcgggacgttatatacaacagatgcttgaccaacgctgccaagagattgctgcagaactctgccaaggcggacttcgtaaaatgtgtgtgccctctagccggatagtagctcgaaacgccgtgggcattactcatcaaaatacacttgaatggagatgctttgatacagcctctttgctggagagcaatcaagaaaacaacggtgttaattgcgtggacgactgtggccacacgataccgtgtcctggcggcgtacaccggcaaaacagtaatcacgcaacgcgccatgagatactgtccaaattggtcgaagaaggagtacaacggttctgcagtccttatcaagcatctgccaacaagtactgtaacgacaaatttccagggaccattgcgaggaggtcgaagggcttcggaaacaatgtcgaggttgcgtggaggtgttacgagaaggccagcttgctgtactcggtttatgctgagtgtgcgagcaactgcggaacaacgtggtactgccctggaggacgacgagggacgtcgacagaactagacaagcggcattatacagaagaggaaggaattcgccaggcaatcggatccgtcgacagcccatgttctgaagttgaagtctgcctaccgaaggatgagaatcccccggtgtgtttagatgaaagtggccagatttcacgaactggtggtgggccaccgtcacaaccgcctgagatgcaacagcccgccgatcgttcggacgagagaggtggcggtaaggaacagtcgcctggaggagaagctcagccggaccatccaacgaagggtggtaacatagacctgcctgagaaatcaacatctcccgagaagacgccgaaaaccgagatccatggtgacagcacgaaagcgacgctcgaagaggggcagcaactaacgctcacgtttatctccactaaactggatgttgctgtaggctcgtgtcattcactcgtcgcgaatttccttgatggatttttgaagtttcagacgggctcaaattcggcgttcgatgtggtagaagtggaagagccagcaggacccgcagtgcttacgataggtctgggacacaaaggccgtctcgctgttgtcctcgactacaccaggctcaatgctgctttaggatcagctgcttacgtggtcgaagattctggatgcagctcaagtgaagaggttagtttccaaggagtgggtagtggagcgacgctcgtggtgacgacgcttggcgagagtcctacggccgtctctgcttgatttatagtactctttggagcatgcttgtggaggaacgggacaatctcggcaaaatcaggatgaagtttgtgagatacagatcgttcctgaacagtggaagatgcgtcactattacacctatatgcgtcctggttcttgtagagttggagttcttgcaggtgtaatgactatgacatacggatataacttcatacggggaactgtg

SEQ ID NO: 4 - DNA, 48 bp, Toxopolasmosis gondii
actgtggtctctaggtatggaagcatatggagaagcgtcgcattctca

SEQ ID NO: 5 - DNA, 49 bp, Toxopolasmosis gondii
actgttctagatcagagcgttagttgctgcccctcttcgagcgtcgctt

SEQ ID NO: 6 - protein, 198 aa, Toxopolasmosis gondii
MALSSLNNIRPFSGLLGCGLLFGALVVVVACVFSVPVEAGVLRKVAGAGSLQASIGEHDFFNDYDQDEEYRKRQQELQNQSPEEVEEAKRKYHEELRRKAEEDAETKRKQEAVIQELKEVAKKRGLREAAEREEKRIDEQQANYEQRQQELRDMDSAMEERLMQQRKKDQEERELARKNSDKVMEELKEKLARRRKSM

SEQ ID NO: 7 - protein, 198 aa, Toxopolasmosis gondii; identical to SEQ ID NO: 6

SEQ ID NO: 8 - DNA, 960 bp, Toxopolasmosis gondii
ttgtcggatagaacacatcaaaaattttttctgtttcatctgtcacgtgcgtccttttggtggaagcgacgcgtcgtcgcggccctgttgggggtagtcaatatttcagtaagcgtttctagcgacacccgctacacagaacactcggttgaagcactgtgatgctggcgtttctgtccgctgtctttctgcagaatggcgctttcttctttgaacaatatcaggccttttagcgggttgctgggttgcggcctgctgtttggcgcccttgtggtcgtggtggcatgtgttttcagcgttcctgtggaagcaggcgttcttcgtaaggtagcaggtgcaggaagtctccaggcgtctattggagagcacgatttttttaacgattacgatcaggacgaggaatacaggaagcgccagcaagaactgcagaatcagagtccagaagaagtcgaggaagcgaaacgcaaataccacgaagagctgagacggaaagcagaagaagatgcagagacgaaacgtaagcaagaagcagtcattcaagaactgaaagaggtggcaaagaaaagaggacttcgtgaagccgctgagcgtgaggagaagcgcattgatgagcagcaggctaattacgagcaacgacaacaagaactgagagacatggattcagcaatggaggagaggcttatgcagcagagaaaaaaagaccaggaagagagagaacttgcaagaaaaaacagcgataaggtcatggaggagctcaaagagaaactcgcaagacgcaggaaatcaatgtagaagaaaggcaagttctgactagtgtatgaagtgtagcagcggtccgttattaccgtgtatacagggagatcgtcgttcagtttgaagtgtttattccgtgttgaaagaagcgtttgtgtaatgcagatgatcctgagatgatagtgcgggaaatcgaatgactcattg

SEQ ID NO: 9 - DNA, 41 bp, Toxopolasmosis gondii
actgtggtctctaggtatggcgctttcttctttgaacaata

SEQ ID NO: 10 - DNA, 38 bp, Toxopolasmosis gondii
actgttctagatcacattgatttcctgcgtcttgcgag

SEQ ID NO: 11 - protein, 236 aa, Toxopolasmosis gondii
MARHAIFFALCVLGLVAAALPQFATAATASDDELMSRIRNSDFFDGQAPVDSLRPTNAGVDSKGTDDHLTTSMDKASVESQLPRREPLETEPDEQEEVHFRKRGVRSDAEVTDDNIYEEHTDRKVVPRKSEGKRSFKDLLKKLALPAVGMGASYFAADRILPELTEQQQTGEEPLTTGQNVSTVLGFAALAAAAAFLGMGLTRTYRHFSPRKNRSRQPALEQEVPESGKDGEDARQ

SEQ ID NO: 12 - protein, 236 aa, Toxopolasmosis gondii; identical to SEQ ID NO: 11

SEQ ID NO: 13 - DNA, 1120 bp, Toxopolasmosis gondii
ttactttcttcggattacattcttccactaaaagctggttttgtccagtatccattcgtcgctaccgttgcgcagtcacgttgaattttgcagcggcaaaacatcttgtgtaaaattcgagttttgttgatgattgaagtaccctgtattggggcttgctaacgttttgtattaaaagggtttactgcggcgtctcatttccaaaatggcccgacacgcaatttttttcgcgctttgtgttttaggcctggtggcggcggctttgccccagttcgctaccgcggccaccgcgtcagatgacgaactgatgagtcgaatccgaaattctgactttttcgatggtcaagcacccgttgacagtctcagaccgacgaacgccggtgtcgactcgaaagggaccgacgatcacctcaccaccagcatggataaggcatctgtagagagtcagcttccgagaagagagccattggagacggagccagatgaacaagaagaagttcatttcaggaagcgaggcgtccgttccgacgctgaagtgactgacgacaacatctacgaggagcacactgatcgtaaagtggttccgaggaagtcggagggcaagcgaagcttcaaagacttgctgaagaagctcgcgctgccggctgttggtatgggtgcatcgtattttgccgctgatagaattctgccggaactaacagagcagcaacagacaggcgaagaacccctaaccaccggccagaatgtgagcactgtgttaggcttcgcagcgcttgctgctgccgcagcgttccttggcatgggtctcacgaggacgtaccgacatttttccccacgcaaaaacagatcacggcagcctgcactcgagcaagaggtgcctgaatcaggcaaagatggggaggatgcccgccagtaggatatgggggctaataaaagtgagtaggagctcgaggacagtgtcccgaacgcgcctgagaggcagacagacacagaagagtgaagaaaaacaacatggtattacgtgcggtgagtgtttgctgtcacgtgttttttgcgccacaaagacagcttgtgttgtatgcatgggatcgacagttcatggacggcgctacccagagag

SEQ ID NO: 14 - DNA, 37 bp, Toxopolasmosis gondii
actgtgaggactcaggtatggctttgccccagttcgc

SEQ ID NO: 15 - DNA, 35 bp, Toxopolasmosis gondii
actgttctagatcactggcgggcatcctccccatc

SEQ ID NO: 16 - DNA, 324 bp, Toxopolasmosis gondii
atgggtcatcaccatcatcatcacgggtccctgcaggactcagaagtcaatcaagaagctaagccagaggtcaagccagaagtcaagcctgagactcacatcaatttaaaggtgtccgatggatcttcagagatcttcttcaagatcaaaaagaccactcctttaagaaggctgatggaagcgttcgctaaaagacagggtaaggaaatggactccttaagattcttgtacgacggtattagaattcaagctgatcaggcccctgaagatttggacatggaggataacgatattattgaggctcaccgcgaacagattggaggt

SEQ ID NO: 17 - protein, 108 aa, Toxopolasmosis gondii
MGHHHHHHGSLQDSEVNQEAKPEVKPEVKPETHINLKVSDGSSEIFFKIKKTTPLRRLMEAFAKRQGKEMDSLRFLYDGIRIQADQAPEDLDMEDNDIIEAHREQIGG

SEQ ID NO: 18 - protein, 456 aa, Toxopolasmosis gondii; identical to SEQ ID NO: 1

SEQ ID NO: 19 - protein, 456 aa, Toxopolasmosis gondii; identical to SEQ ID NO: 1

SEQ ID NO: 20 - protein, 456 aa, Toxopolasmosis gondii; identical to SEQ ID NO: 1

SEQ ID NO: 21 - protein, 456 aa, Toxopolasmosis gondii; identical to SEQ ID NO: 1

SEQ ID NO: 22 - protein, 456 aa, Toxopolasmosis gondii
MGQALFLTVLLPVLFGVGPEAYGEASHSHSPASGRYIQQMLDQRCQEIAAELCQSGLRKMCVPSSRIVARNAVGITHQNTLQWRCFDTASLLESNQENNGVNCVDDCGHTIPCPGGVHRQNSNHATRHEILSKLVEEGVQRFCSPYQASANKYCNDKFPGTIARRSKGFGNNVEVAWRCYEKASLLYSVYAECASNCGTTWYCPGGRRGTSTELDKRHYTEEEGIRQAIGSVDSPCSEVEVCLPKDENPPVCLDESGQISRTGGGPPSQPPEMQQPADRSDERGGGKEQSPGGEAQPDHPTKGGNIDLPEKSTSPEKTPKTEIHGDSTKATLEEGQQLTLTFISTKLDVAVGSCHSLVANFLDGFLKFQTGSNSAFDVVEVEEPAGPAVLTIGLGHKGRLAVVLDYTRLNAALGSAAYVVEDSGCSSSEEVSFQGVGSGATLVVTTLGESPTAVSA

SEQ ID NO: 23 - protein, 456 aa, Toxopolasmosis gondii
MGQALFLTVLLPVLFGVGPEAYGEASHSHSPASGRYIQQMLDQRCQEIAAELCQSGLRKMCVPSSRIVARNAVGITHQNTLQWRCFDTASLLESNQENNGVNCVDDCGHTIPCPGGVHRQNSNHATRHEILSKLVEEGVQRFCSPYQASANKYCNDKFPGTIARRSKGFGNNVEVAWRCYEKASLLYSVYAECASNCGTTWYCPGGRRGTSTELDKRHYTEEEGIRQAIGSVDSPCSEVEVCLPKDENPPLCLDESGQISRTGGGPPSQPPEMQQPADRSDERGGGKEQSPGGEAQPDHPTKGGNIDLPEKSTSPEKTPKTEIHGDSTKATLEEGQQLTLTFISTKLDVAVGSCHSLVANFLDGFLKFQTGSNSAFDVVEVEEPAGPAVLTIGLGHKGRLAVVLDYTRLNAALGSAAYVVEDSGCSSSEEVSFQGVGSGATLVVTTLGESPTAVSA

SEQ ID NO: 24 - protein, 456 aa, Toxopolasmosis gondii; identical to SEQ ID NO: 23

SEQ ID NO: 25 - protein, 456 aa, Toxopolasmosis gondii; identical to SEQ ID NO: 23

SEQ ID NO: 26 - protein, 456 aa, Toxopolasmosis gondii; identical to SEQ ID NO: 23

SEQ ID NO: 27 - protein, 456 aa, Toxopolasmosis gondii
MGQALFLTVLLPVLFGVGPEAYGEASHSHSPASGRYIQQMLDQRCQEIAAELCQSGLRKMCVPSSRIVARNAVGITHQNTLQWRCFDTASLLESNQENNGVNCVDDCGHTIPCPGGVHRQNSNHATRHQILSKLVEEGVQRFCSPYQASANKYCNDKFPGTIARRSKGFGNNVEVAWRCYEKASLLYSVYAECASNCGTTWYCPGGRRGTSTELDKRHYTEEEGIRQAIGSVDSPCSEVEVCLPKDENPPLCLDESGQISRTGGGPPSQPPEMQQPADRSDERGGGKEQSPGGEAQPDHPTKGGNIDLPEKSTSPEKTPKTEIHGDSTKATLEEGQQLTLTFISTKLDVAVGSCHSLVANFLDGFLKFQTGSNSAFDVVEVEEPAGPAVLTIGLGHKGRLAVVLDYTRLNAALGSAAYVVEDSGCSSSEEVSFQGVGSGATLVVTTLGESPTAVSA

SEQ ID NO: 28 - protein, 456 aa, Toxopolasmosis gondii
MGQALFLTVLLPVLFGVGPEAYGEASHSHSPASGRYIQQMLDQRCQEIAAELCQSGLRKMCVPSSRIVARNAVGITHQNTLQWRCFDTASLLESNQENNGVNCVDDCGHTIPCPGGVHRQNSNHATRHEILSKLVEEGVQRFCSPYQASANKYCNDKFPGTIARRSKGFGNNVEVAWRCYEKASLLYSVYAECASNCGTTWYCPGGRRGTSTELDKRHYTEEEGIRQAIGSVDSPCSEVEVCLPKDENPPLCLDESGQISRTGGGPPSQPPEMQQPADRSDERGGGKEQSPGGEAQPDHPTKGGNIDLPEKSTSPEKTPKTEIHGDSTKATLEEGQQLTLTFISTKLDVAVGSCHSLVANFLDGFLKFQTGSNSAFDVVEVEDPAGPAVLTIGLGHKGRLAVVLDYTRLNAALGSAAYVVEDSGCSSSEEVSFQGVGSGATLVVTTLGESPTAVSA

SEQ ID NO: 29 - protein, 456 aa, Toxopolasmosis gondii; identical to SEQ ID NO: 22

SEQ ID NO: 30 - protein, 456 aa, Toxopolasmosis gondii; identical to SEQ ID NO: 22

SEQ ID NO: 31 - protein, 456 aa, Toxopolasmosis gondii; identical to SEQ ID NO: 1

SEQ ID NO: 32 - protein, 456 aa, Toxopolasmosis gondii; identical to SEQ ID NO: 23

SEQ ID NO: 33 - protein, 456 aa, Toxopolasmosis gondii; identical to SEQ ID NO: 23

SEQ ID NO: 34 - protein, 198 aa, Toxopolasmosis gondii; identical to SEQ ID NO: 6

SEQ ID NO: 35 - protein, 198 aa, Toxopolasmosis gondii; identical to SEQ ID NO: 6

SEQ ID NO: 36 - protein, 198 aa, Toxopolasmosis gondii; identical to SEQ ID NO: 6

SEQ ID NO: 37 - protein, 198 aa, Toxopolasmosis gondii; identical to SEQ ID NO: 6

SEQ ID NO: 38 - protein, 198 aa, Toxopolasmosis gondii; identical to SEQ ID NO: 6

SEQ ID NO: 39 - protein, 198 aa, Toxopolasmosis gondii; identical to SEQ ID NO: 6

SEQ ID NO: 40 - protein, 198 aa, Toxopolasmosis gondii; identical to SEQ ID NO: 6

SEQ ID NO: 41 - protein, 198 aa, Toxopolasmosis gondii; identical to SEQ ID NO: 6

SEQ ID NO: 42 - protein, 198 aa, Toxopolasmosis gondii
MALSSLNNIRPFSGLLGCGLLFGALVVVVACVFSVPVEAGVLRKVAGAGSLQASIGEHDFFNDYDQDEEYRKRQQELQNQSPEEVEEAKRKYHEELRRKAEEDAETKRKQEAVIQELKEVAKKRGLREAAEREEKRTDEQQANYEQRQQELRDMDSAMEERLMQQRKKDQEERELARKNSDKVMEELKEKLARRRKSM

SEQ ID NO: 43 - protein, 198 aa, Toxopolasmosis gondii
MALSSLNNIRPFSGLLGCGLLFGALVVVVACAFSVPVEAGVLRKVAGAGSLQASIGEHDFFNDYDQDEEYRKRQQELQNQSPEEVEEAKRKYHEELRRKAEEDAETKRKQEAVIQELKEVAKKRGLREAAEREEKRTDEQQANYEQRQQELRDMDSAMEERLMQQRKKDQEERELARKNSDKVMEELKEKLARRRKSM

SEQ ID NO: 44 - protein, 167 aa, Toxopolasmosis gondii
MLVFLSAVFLQNGAFFFEQYQASIGEHDFFNDYDQDEEYRKRQQELQNQSPEEVEEAKRKYHEELRRKAEEDAETKRKQEAVIQELKEVAKKRGLREAAEREEKRIDEQQANYEQRQQELRDMDSAMEERLMQQRKKDQEERELARKNSDKVMEELKEKLARRRKSM

SEQ ID NO: 45 - protein, 198 aa, Toxopolasmosis gondii; identical to SEQ ID NO: 6

SEQ ID NO: 46 - protein, 198 aa, Toxopolasmosis gondii; identical to SEQ ID NO: 6

SEQ ID NO: 47 - protein, 198 aa, Toxopolasmosis gondii; identical to SEQ ID NO: 6

SEQ ID NO: 48 - protein, 198 aa, Toxopolasmosis gondii; identical to SEQ ID NO: 6

SEQ ID NO: 49 - protein, 198 aa, Toxopolasmosis gondii; identical to SEQ ID NO: 6

SEQ ID NO: 50 - protein, 383 aa, Toxopolasmosis gondii
MRGGTSALLHALTFSGAVWMCTPAEALPIQKSVQLGSFDKVVPSREVVSESLAPSFAVTETHSSVQSPSKQETQLCAISSEGKPCRNRQLHTDNGYFIGASCPKSACCSKTMCGPGGCGEFCSSNWIFCSSSLIYHPDKSYGGDCSCEKQGHRCDKNAECVENLDAGGGVHCKCKDGFVGTGLTCSEDPCSKRGNAKCGPNGTCIVVDSVSYTCTCGDGETLVNLPEGGQGCKRTGCHAFRENCSPGRCIDDASHENGYTCECPTGYSREVTSKAEESCVEGVEVTLAEKCEKEFGISASSCKCDNGYSGSASATSHHGKGESGSEGSLSEKMNIVFKCPSGYHPRYHAHTVTCEKIKHFALDGAGNHDTTTYVARRRYPASL

SEQ ID NO: 51 - protein, 249 aa, Toxopolasmosis gondii
YHPDKSYGGDCSCEKQGHRCDKNAECVENLDAGGGVHCKCKDGFVGTGLTCSEDPCSKRGNAKCGPNGTCIVVDSVSYTCTCGDGETLVNLPEGGQGCKRTGCHAFRENCSPGRCIDDASHENGYTCECPTGYSREVTSKAEESCVEGVEVTLAEKCEKEFGISASSCKCDNGYSGSASATSHHGKGESGSEGSLSEKMNIVFKCPSGYHPRYHAHTVTCEKIKHFALDGAGNHDTTTYVARRRYPASL

SEQ ID NO: 52 - DNA, 3837 bp, Toxopolasmosis gondii
tcttctcttcttccgtacttttccctgcatttcacacccctggtatgactccacaccgcgtgtaaatgtcccttaggtgacacccgcagcagcgcgtaggaggaagtagatgtcagtgtagacgtttttgagatgagagacgataacgtaaaatgccgccgataacttctgcattatacacactctctctccacgcctaggatgacaggtacggcggcacacggaggaaagtgggggggggggggggggcgaacagaaaggtcacatggaaggccgctcgactctccactcacgaagtgaaggcttcgtcccgttttgctggacaacgaatgcgaacttcttcactcgcttgtgacacacacaactccagaggcacagagatgtgaagcagaagagtggcgtgtgcgtcgcttctgtcggcggcaagccccgctccgtctctttggtggcgattctggtgtgcaccgtgtgccaagaagttgcgtgtcacgcgacttttggaaatgcatcaggttcagagtcgttatgttgcgattcaggctctcggcagagaatcatttccctgtaagctagttgaactcgcctttttaaaagcggcagcagtgcccttgtggaaggcctcactgtgcctactttcctcgtcctgagtttttccgccttcggcctcattttttgctcaccaaaatcgtgtcctaccgtcaagttttgccatagactcctacgggaaaaaacaagccggtcgacacggacgacgcccgcagggaagcgtcccctccgcagaaatcgggagacaactgtcgttgacggtgctgcgcgaaaggtcacagagtttccagtgtgttcatcagacctcactgtgcactgttagcggccgctgtcccgcctggtcaacaagtatcacaccctcgtccccgccattggcacggagctcgatgagctgcagtgtcgcttttaggggagtcgtgcaatcacgccgcaacacaggcgtgattcgatcttcaattgctaggtaaccactcgtgcttggtagctctgcaatggctcgagcgacgggggtgatgcaacatgctgctaaaaactcgacagacgtgtcaccggaacccacctaaataggagaccacgggtctctggtgtgtcgcgtcgcattctcgcgtcgcattctcgcgtcgcaatgaccggccagttgctcgacgtcgccagccgggactgaagagcgttcatcgagtcagcagcattgcgtccccttgctcggtgaaaaaagactctctggtcgagtctagctcgtgtcacttctgtttctaacctccttcgttcaccggtacacctccgatgtgacttttggtacacttgccctgtcgcacgacgcacgctgtcactcaacttgctgctagcgcaatcgataggttccctcgaaccagccatcacacacacaccttttccgggaagacgtttgcgggcggtgggtcgcagctcgtcgagagtgcgtttctgtgcatttctgtgggcagtgcagcgcgtttgcgcgccttactctgtgtgtaacttccttgtccaacactggtaaaaatgcgaggcgggacgtccgcgctgttgcacgcgctcaccttcagtggggccgtgtggatgtgcaccccagcggaggctttgccgattcagaagtctgtgcagctgggcagctttgacaaagttgtgccgagccgcgaagtcgtctctgagagtcttgctccgtctttcgcggtgactgagactcactcgtctgtgcaatcccccagcaagcaggagacgcaactctgtgctatctcgagtgaaggcaagccatgtcgaaaccgtcagttgcacactgacaacgggtacttcatcggggccagttgccccaagagcgcttgctgcagcaagaccatgtgcggccccggcggctgcggagaattctgctccagcaactggattttttgcagcagttcgctcatctaccatcctgacaaaagctatggaggagactgcagctgtgaaaagcagggccatcggtgcgacaaaaacgcagaatgcgtcgaaaacttggacgcgggtgggggtgtgcactgcaagtgcaaagacggcttcgtcggcactgggttgacttgctccgaggatccttgttcaaaaagagggaacgcgaagtgcggacccaacgggacgtgcatcgtcgtcgattcagtcagctacacatgcacctgcggcgacggcgaaactctagtgaacctcccggaagggggacaaggatgcaagaggactggatgtcatgccttcagggagaactgcagccctggtagatgtattgatgacgcctcgcatgagaatggctacacctgcgagtgccccacagggtactcacgtgaggtgacttccaaggcggaggagtcgtgtgtggaaggagtcgaagtcacgctggctgagaaatgcgagaaggaattcggcatcagcgcgtcatcctgcaaatgcgataacggatactccggatctgcttccgcaacctcccaccatgggaaaggagaatcgggatccgaggggagcttgagtgaaaaaatgaatattgtcttcaagtgccccagtggctaccatccaagataccatgcccacaccgtgacgtgtgagaaaattaagcactttgcccttgacggggccggcaaccacgacacgactacgtatgtcgcaagacgaaggtacccagcgagtctctgagagcggagatcagcgcaaagacaagatgcagagtttgactcgagaaacaatagtaacacgaagtaaaaagtctccacactaagccaaggattgagaatatttcgatttgtgccgctggcaatagtggccttggcctagaaagaagttctgcaacgaagcgatcggctcacacgcggatacacagatgggtttgtaccgagaacgttaggtttgtgaaccgagttcaggtaaaacaaagtagattgtgcctttacgcagacagcgagggaaaacatgaggacacactgccaactaaagcaagactgcctcactaattaccaccgacacacgacatggttacccccgcgttttgccgcgtgcaaagtttgaattctgatggttctcgagtctgaaagcctaaaccgcccaaccatgtatgaaataagaacccatcaaacgtgagacatctctgccgaagtgcctacgaaaagaacgcttctgccactaggaggtgcggcctcttcattctatgagaacctgctttgtcggtgtcaacctctggggaaatcgcctgcctttacacattttgctcgttgtagagcaagggatctgttgctgcgtttactccaatacaatgatcgccgtttcgctgtaggcaagcgatccgaaaatgtacgttcgagtcagcagctacttgagaagcagccaacgccgacacttgctgcgtttgactgaggtgcactcgcaaacagtctcgtctccccggggcaatttctgagagaaatgcgggaatggacgtaatggtgctcttctgtgagtgctcttccaccaatttttcgacaagtgttttcgtgacagtcgagtataccttcttatgtcattctgtctccgtcagtgctatcggattcttcctattcctctaccctttctacagtcgcatacaaagctgctgaaacaagacttcctttgtctagggtagttgtacactccacacatatctgactgaaacctacggcaggaagtctggtcggcactgtgcttccttgttggcttttcgtcgtttctttgtctacgagcttcactgggtccttgacacggcttgtgagcgttgtgctcaatattcgaccagctgtatttgtg

SEQ ID NO: 53 - DNA, 53 bp, Toxopolasmosis gondii
actgtggtctctaggtatgatctaccatcctgacaaaagctatggaggagact

SEQ ID NO: 54 - DNA, 39 bp, Toxopolasmosis gondii
acttgttctagatcagagactcgctgggtaccttcgtct

SEQ ID NO: 55 - protein, 580 aa, Toxopolasmosis gondii
MRASLPVHLVVCTQLSAVWFGVAKAHGGHRLEPHVPGFLQGFTDITPAGDDVSANVTSSEPAKLDLSCVHSDNKGSRAPTIGEPVPDVSLEQCAAQCKAVDGCTHFTYNDDSKMCHVKEGKPDLYDLTGGKTASRSCDRSCFEQHVSYEGAPDVMTAMVTSQSADCQAACAADPSCEIFTYNEHDQKCTFKGRGFSAFKERGVLGVTSGPKQFCDEGGKLTQEEMEDQISGCIQLSDVGSMTADLEEPMEADSVGACMERCRCDGRCTHFTFNDNTRMCYLKGDKMQLYSSPGDRTGPKSCDSSCFSNGVSYVDDPATDVETVFEISHPIYCQVICAANPLCTVFQWYASEAKCVVKRKGFYKHRKTGVTGVTVGPREFCDFGGSIRDREEADAVGSDDGLNAEATMANSPDFHDEVECVHTGNIGSKAQTIGEVKRASSLSECRARCQAEKECSHYTYNVKSGLCYPKRGKPQFYKYLGDMTGSRTCDTSCLRRGVDYSQGPEVGKPWYSTLPTDCQVACDAEDACLVFTWDSATSRCYLIGSGFSAHRRNDVDGVVSGPYTFCDNGENLQVLEAKDTE

SEQ ID NO: 56 - protein, 173 aa, Toxopolasmosis gondii
SEPAKLDLSCVHSDNKGSRAPTIGEPVPDVSLEQCAAQCKAVDGCTHFTYNDDSKMCHVKEGKPDLYDLTGGKTASRSCDRSCFEQHVSYEGAPDVMTAMVTSQSADCQAACAADPSCEIFTYNEHDQKCTFKGRGFSAFKERGVLGVTSGPKQFCDEGGKLTQEEMEDQISG

SEQ ID NO: 57 - DNA, 3121 bp, Toxopolasmosis gondii
ttttctgtgcatctgtgctgcaaaacgggcctctgtgcattatttccccaccaacaattgccgcgtcgatccgggtcccgctcaagctctgcagaactaggctctcgatatagatcagtacaatcattcgcttctgacaatcgcatcgactgagcgacgcgttgatcgtcgactgtcgtgcgtcgcattcgggcatctcgaaccggtgttgattccctgtgtcattatttcacttccgtccttctctcgtggcgatctataatacgcgtgtgttgttgcgtgcattgcttgtgttgttgtggatgtgttttcttttgtgaccgctcacgaacaccccacgcaaaatgagagcgtcgctcccggttcacctcgttgtgtgcacgcagctaagtgccgtttggtttggagtggctaaagcccatggtggacaccgactggaaccgcatgttcccggattcctgcaaggcttcactgatatcacgcctgcaggtgatgacgttagtgccaacgtaacaagttcggagcctgcaaaacttgatctctcttgtgtgcactctgacaataagggatcaagggctcccacaataggcgagccagtgccagatgtgtccctggaacaatgtgctgcgcaatgcaaggctgttgatggctgcacacatttcacttataatgacgattcgaagatgtgccatgtgaaggagggaaaacccgatttatacgatctcacaggaggcaaaacagcatcgcgcagttgcgatagatcatgcttcgaacaacacgtatcgtatgagggagctcctgacgtgatgacagcgatggtcacgagccagtcagcggactgtcaggctgcgtgtgcggctgacccgagctgcgagatcttcacttataacgaacacgaccagaaatgtactttcaaaggaagggggttttctgcgtttaaggaacgaggggtgttgggtgtgacttccgggccgaaacagttctgcgatgaaggcggtaaattaactcaagaggagatggaagatcagatcagtggctgcattcaattgagtgacgttggatcaatgactgctgacctggaggagcctatggaggctgattctgttggcgcttgtatggaacggtgccgctgtgatggaagatgcacgcacttcacgttcaacgataatactcggatgtgctacctcaaaggtgacaagatgcagttgtactcatctccaggtgacagaaccggcccaaagagctgcgattcaagctgcttctcgaacggggtttcttacgtcgatgatccggcgacagatgttgagaccgtattcgaaatttcacacccaatttattgtcaagtaatctgcgccgcaaatccgttgtgtacagtgtttcagtggtatgcctccgaggcaaagtgcgtcgtcaagagaaaggggttttacaaacacagaaaaacaggtgtcacgggagtcacagtgggccctcgggagttctgcgattttggcggtagcatccgcgaccgagaagaggcagacgccgttggatcagacgatggcctcaacgcggaagcaactatggcaaattctcctgattttcacgacgaagtagaatgcgtccacacgggcaacattgggtcaaaagcacaaaccattggagaagtgaaacgcgcaagtagtttgagtgagtgcagagccagatgccaagcggagaaagaatgcagccactacacttacaatgtaaaatccggtttgtgttatccaaaaagaggaaagcctcaattttataagtatcttggcgacatgacgggatccagaacatgtgatacaagttgccttaggaggggagtcgattactcacagggccctgaagtaggaaagccttggtattctacgctgccgacagactgccaagttgcatgcgacgctgaggatgcttgcctggtgttcacctgggattcggcgacgtcacgatgctacctcatcggctcaggtttctcggcacatcgacggaacgacgtggatggcgtggtatctggaccctatactttctgtgacaatggcgaaaaccttcaggtgcttgaagcgaaagacacagaatgacccaggagggtgccagatactttgtgtgactgcgacatgcagtcatgtactcaaagtgttgtacatggacaggaggactttttttttaagtcattgcagaggtgcgttttcggagcagcactataactgcgtcagcgactaagcacgccacgtagctgaatgaaacgcagccaccttcgtgtatgtatgcttcgttttttgtcgctgtgcagttttgaatcatttcccttatgggacatttctgaaaaatgctccccgttcgcttgtagcactatgagaggggccgaagactgcaatggaggtagcgctgcgttgaaaagacgaggcgctacatttcgcgtagcgacaaggccgtgtagagttttgcttttcgcgagacactgctctgagtgtcatatgcatcaaatgcagtggtagcacacagaggtgagaagaatgatcacctgcgggggaatggctttgctaaacaacaaggtcgctgtgtgactttacacaacgaaactactgtggtgagtgctcagttgagtgaaaagaaatgccgcgttatcgtgagttctggttcggtggactttgccaccgtagtaaaactcaacctgtaacggaatgcccagttttactgctctctttaaagggcgtccacgttctctatattcaagctgtttacccacctgcgtttcggtgcatcgcgcgtgccacatcaaaaatccaggtaacggtgcgggacctatgctacactttatatctctcagaaagcatacacccactgattatggacaacgctgtggtcgcgttgtaccacaatgcaggaatactcagttcaccttgcaagtgttctggtgttcattgcgtgtcagaagtacacgaaaagagacttctttggcctccaagtgatacgtaaccgcggcagtcatgaacagagtcactcgtgcttctgaaacgcacgtcttctgtacagagacagatgcagtgtgcatacaggaagcccctcgattgttgccgtagcaggtagccagtagaagaaacaaagacacggt

SEQ ID NO: 58 - DNA, 54 bp, Toxopolasmosis gondii
actgtggtctctaggtatgagttcggagcctgcaaaacttgatctctcttgtgt

SEQ ID NO: 59 - DNA, 47 bp, Toxopolasmosis gondii
actgttctagatcagccactgatatgatcttccatctcctcttgagt

SEQ ID NO: 60 - protein, 349 aa, Toxopolasmosis gondii
MRLFRCCAAAVVAAESLLWLKNGSPFFAFLPGNGEIADNCSGNPCGGTAAGTCINTPSGYDCRCEPGYVLGVENDQVTCMMPSGVPMANFVQLSEKPAACSSNPCGPEAAGTCNETNSGYICRCNQGYRISLDGTGNVTCIVRQESGCEENGCGPPDAVQSCRRLTGTAGRLCVCKENFIATIDASAHITCKRVPPHYRKPPFEFGKGGHPVDSEPSKRQREDEGESREPESDSTEPGRDQERRTPLEESQEPEGSTPDSQQSRGGSGSDSTESEEQGKEREEGSGHAGAIAGGVIGGLLLLSAAGAGVAYMRKSGSGGGEEIEYERGIEAAEASEVEVLVDLDSKTWD

SEQ ID NO: 61 - protein, 326 aa, Toxopolasmosis gondii
SPFFAFLPGNGEIADNCSGNPCGGTAAGTCINTPSGYDCRCEPGYVLGVENDQVTCMMPSGVPMANFVQLSEKPAACSSNPCGPEAAGTCNETNSGYICRCNQGYRISLDGTGNVTCIVRQESGCEENGCGPPDAVQSCRRLTGTAGRLCVCKENFIATIDASAHITCKRVPPHYRKPPFEFGKGGHPVDSEPSKRQREDEGESREPESDSTEPGRDQERRTPLEESQEPEGSTPDSQQSRGGSGSDSTESEEQGKEREEGSGHAGAIAGGVIGGLLLLSAAGAGVAYMRKSGSGGGEEIEYERGIEAAEASEVEVLVDLDSKTWD

SEQ ID NO: 62 - DNA, 3394 bp, Toxopolasmosis gondii
cagtccggagcacactcctacaataaacttgatacgtgtcattttgtgaaacgacacagcacataaccactcggactgtctcacgaagctgtagggcggattcaccaatgatctttcgcagccgatccaaaactacttgcccacttccggtgtacgtacatcgcgcgacatgagaggcattcattgttttccatagaaaacactactggacaaccattcggtagcgcacaagttgagcctctgacaaatctttcctcatcacgtgaatacacgctgcgtgattcgtcagtgactccactgtggtctttaaccaccatcagagtcctgtaagcatcctttgtttccgtttaaaatgcctgccagatggcacgacgccgtctggttttgccggctttctccgagtcctattagactttgatgccttacggcttttttttaagaatggttcttttgagatttgccgactttccagttccgccaccagacgctcctgttgaactgccaccggcacgatgcagtattccgccacgaaaacgcgcaccgcaagctccgctaccattaaacgggtttcgtctgctttagatgtttccttccgcgtcatcaaggcaaaagcattgccactgatgttaccgaagctttcccgccatgctgcgcacaatgcccaatcttccgtcacggacctcttccggtaaccacctaaaggaggattactgggcaacccaaaacgctgcaacaagaagcacagtccaggtgtcgctagattcgagcctgcatggtcgttccgtagctccatacaacaattctctgtgtgacggcgagaggagtaacgcgctagtgtgtgtcagcgacgcggcagtcgatccgatcctgcaacaggcagaggtgtgtcgatgctcagtgatgcgacggcgtatctgaagaggactgtagctccaccacgaccttcgtgggagcacgaagtgtactctgttgtcgtcggtctcgtatttttttgagttgtgtacttcgctgcaagaggagggtgagattcgacatctgtgggcgtttgggatcgtgatgacatcgactgtgctttgatatatgatgtgttttttttcgattggatgagcacattccagtaagcttcctgccgcgcgtctctgctatgaggctcttccggtgctgtgctgcggccgttgtggcggccgaatcgttactgtggctgaagaacggctccccgttttttgcctttcttcctgggaatggagagattgcagacaactgctctgggaatccatgcggtggcaccgcagctggtacgtgcataaacacaccatctggatatgattgcaggtgcgaaccaggctacgttctgggcgttgaaaatgaccaggtcacgtgcatgatgccctcaggtgtacccatggctaattttgtacagctgtcggaaaagcctgcagcttgcagctcaaacccttgtggacctgaggcagccggcacctgcaacgagacaaacagtggttacatttgccgctgtaatcaaggctacagaatatctctcgacgggacaggaaacgtgacatgtattgtaagacaggaaagcggctgtgaggaaaacgggtgtgggccgccagatgcagtacagagttgccgccgactaacagggacggcaggtcgactatgtgtatgcaaggaaaactttatagcgacaatcgacgccagtgcccatatcacctgcaagcgtgtgcctccccattataggaagcctcccttcgaatttggcaagggaggtcatcctgtggactcagaaccatcgaaacgccagagggaagatgaaggtgaaagtcgtgagcctgaaagcgactcaacagaaccggggagagatcaggaaagaagaacaccacttgaggaaagccaggaaccggaaggaagcaccccggacagtcagcagagccgaggtggttctggtagcgacagtaccgagagcgaggaacaaggaaaggagagagaggaaggaagtggacatgctggtgcgatcgctgggggagttattggaggcctgttacttctgagcgctgccggagcgggtgttgcatacatgagaaagagtgggagcggtggaggggaggagatagaatacgagaggggtatcgaggctgcagaggccagtgaagtcgaagtcctcgttgatttggatagcaaaacatgggattaacacgttctcggctgagacttcacaatgtagggtgtcgctggcagatcagctgcaatgcgagaggtgacgcgagtagtgagcaccgcttcttttaagcgcggacattgtgctcggtcttctgtcacccccgaatcaaaacacatgtatgataatagttcctgttgacttcccctgccgacaaagaactgctgtgtcgaggccggcttctgtgcactcatcccaaatgagatggactgatgttttagagacacctcatcgccgacggaaaccatcagctcccagagaaactatgctgcgtcgttttttaggtgatctgttgcgtaatgcgcaccttcatatcatctgtgtgttgactgtttggtcgttttccgtttagtcaaatgaatgcagtgaaatgcagggaatttagcagacaccgagaactgtcctcttgttctgtgcgcgagttgtttttaacgtatagcgatgcgtttgcacttgatattaccctaagccatcagtgggtatttagaggagcccacaggtgatgggggtgatccctgtttcttgtcatttggcttgtagggttcgctggaactatctggtgtcacggaagagtggctttactgtctgtccccaaacgcaaggcatcagtgtaaccccgataggactctggagacttctgcttcactgccgcgttgcaattttcccgcgtcatgtggcaataacggtaattccacgtgcacgccgcataccggatctttgctcccaggctttcttatgaggtcggcatacgtacagcggcggcgtacctccgctctagagaagaccggtccaaccgactttgaacagcatgcttgtgaatgagtgcttaaacaccctgaagtgatggtggaatgtagcagtctgggacggttgatgcgaggatatcaccattagcatagactaccttgctctttagcgaggcgagacaacttatttaggtagccatgaaacacctcgatagtatcaatgacgacgtgcggttcaccaacttccgtcgctagcgcagaaaacagtcggaaacacaactcggtgagcacctgaagtgtcagtacacattcgaccgtcgggacccgggattccgcaagtggcacccgctggtccagtagcaggaacctagttcattcagtataacagatttggggcggcaaagagcaatttgctcgacctaacgcttgc

SEQ ID NO: 63 - DNA, 44 bp, Toxopolasmosis gondii
actgtgtgctctaggtatgtccccgttttttgcctttcttcctg

SEQ ID NO: 64 - DNA, 39 bp, Toxopolasmosis gondii
actgttctagattaatcccatgttttgctatccaaatca